European Patent Application EP 4 332 241 A1, published March 6, 2024. Title: Single nucleotide polymorphism for the prognosis of breast cancer. Applicant: Consejo Superior de Investigaciones Cientificas (CSIC). The sequence listing filed with the application follows.

SEQUENCE LISTING (13 sequences)

SEQ ID NO: 1 - DNA, 194 bp, Homo sapiens
  source 1..194: mol_type = genomic DNA
aatcccttcagttttagctaccaacggccaggaaaagccctcatcttctctttctctcctcagtttacatcttgttggtacctttctagccttagacaaatgatcaccatgttagccttagacgaagaagctggctagtcctttctgtgaagctaatacaatggtcatttccagacaaatttaaaggaaacact

SEQ ID NO: 2 - DNA, 23 bp, synthetic construct
  source 1..23: mol_type = other DNA; note = forward primer G allele rs8570; note (original language) = cebador directo alelo G rs8570; organism (original language) = construccion sintetica
gatcaccatgttagccttatacg

SEQ ID NO: 3 - DNA, 23 bp, synthetic construct
  source 1..23: mol_type = other DNA; note = forward primer C allele rs8570; note (original language) = cebador directo alelo C rs8570; organism (original language) = construccion sintetica
gatcaccatgttagccttatacc

SEQ ID NO: 4 - DNA, 20 bp, synthetic construct
  source 1..20: mol_type = other DNA; note = reverse primer G and C alleles rs8570; note (original language) = cebador reverso alelos G y C rs8570; organism (original language) = construccion sintetica
agcagccttagtgtttcctt

SEQ ID NO: 5 - DNA, 21 bp, synthetic construct
  source 1..21: mol_type = other DNA; note = forward primer first PCR exon 3 RRAS2; note (original language) = cebador directo primera PCR exon 3 RRAS2; organism (original language) = construccion sintetica
gcaggacaagaagagtttgga

SEQ ID NO: 6 - DNA, 20 bp, synthetic construct
  source 1..20: mol_type = other DNA; note = forward primer second PCR exon 5 RRAS2; note (original language) = cebador directo segunda PCR exon 5 RRAS2; organism (original language) = construccion sintetica
tccatgaacttgtccgggtt

SEQ ID NO: 7 - DNA, 23 bp, synthetic construct
  source 1..23: mol_type = other DNA; note = reverse primer first PCR exon 3 RRAS2 and second PCR exon 5 RRAS2; note (original language) = cebador reverso primera PCR exon 3 RRAS2 y segunda PCR exon 5 RRAS2; organism (original language) = construccion sintetica
tgaagcagccttagtgtttcctt

SEQ ID NO: 8 - DNA, 21 bp, synthetic construct
  source 1..21: mol_type = other DNA; note = forward primer exons 3-4 RRAS2; note (original language) = cebador directo exones 3-4 RRAS2; organism (original language) = construccion sintetica
gcaggacaagaagagtttgga

SEQ ID NO: 9 - DNA, 20 bp, synthetic construct
  source 1..20: mol_type = other DNA; note = reverse primer exons 3-4 RRAS2; note (original language) = cebador reverso exones 3-4 RRAS2; organism (original language) = construccion sintetica
tcattgggaactcatcacga

SEQ ID NO: 10 - DNA, 18 bp, synthetic construct
  source 1..18: mol_type = other DNA; note = forward primer Luciferase; note (original language) = cebador directo Luciferasa; organism (original language) = construccion sintetica
tcaaagaggcgaactgtg

SEQ ID NO: 11 - DNA, 19 bp, synthetic construct
  source 1..19: mol_type = other DNA; note = reverse primer Luciferase; note (original language) = cebador reverso Luciferasa; organism (original language) = construccion sintetica
ggtgttggagcaagatgga

SEQ ID NO: 12 - DNA, 19 bp, synthetic construct
  source 1..19: mol_type = other DNA; note = forward primer 18S rRNA; note (original language) = cebador directo 18S rARN; organism (original language) = construccion sintetica
atccattggagggcaagtc

SEQ ID NO: 13 - DNA, 20 bp, synthetic construct
  source 1..20: mol_type = other DNA; note = reverse primer 18S rRNA; note (original language) = cebador reverso 18S rARN; organism (original language) = construccion sintetica
gctcccaagatccaactacg